European Patent Application EP 4 310 500 A2, published January 24, 2024. Title: METHODS AND COMPOSITIONS FOR THE ACTIVATION OF GAMMA-DELTA T-CELLS. Applicant: American Gene Technologies International Inc. Application Not Yet Assigned. The sequence listing filed with the application follows.

SEQUENCE LISTING (67 sequences)

SEQ ID NO: 1 - DNA, 53 bp, synthetic construct
  misc_feature 1..53: note = FDPS shRNA sequence #1
  source 1..53: mol_type = other DNA
gtcctggagtacaatgccattctcgagaatggcattgtactccaggacttttt

SEQ ID NO: 2 - DNA, 53 bp, synthetic construct
  misc_feature 1..53: note = FDPS shRNA sequence #2
  source 1..53: mol_type = other DNA
gcaggatttcgttcagcacttctcgagaagtgctgaacgaaatcctgcttttt

SEQ ID NO: 3 - DNA, 53 bp, synthetic construct
  misc_feature 1..53: note = FDPS shRNA sequence #3
  source 1..53: mol_type = other DNA
gccatgtacatggcaggaattctcgagaattcctgccatgtacatggcttttt

SEQ ID NO: 4 - DNA, 53 bp, synthetic construct
  misc_feature 1..53: note = FDPS shRNA sequence #4
  source 1..53: mol_type = other DNA
gcagaaggaggctgagaaagtctcgagactttctcagcctccttctgcttttt

SEQ ID NO: 5 - DNA, 116 bp, synthetic construct
  misc_feature 1..116: note = miR30 FDPS sequence #1
  source 1..116: mol_type = other DNA
aaggtatattgctgttgacagtgagcgacactttctcagcctccttctgcgtgaagccacagatggcagaaggaggctgagaaagtgctgcctactgcctcggacttcaaggggct

SEQ ID NO: 6 - DNA, 114 bp, synthetic construct
  misc_feature 1..114: note = miR30 FDPS sequence #2
  source 1..114: mol_type = other DNA
aaggtatattgctgttgacagtgagcgacactttctcagcctccttctgcgtgaagccacagatggcagaagggctgagaaagtgctgcctactgcctcggacttcaaggggct

SEQ ID NO: 7 - DNA, 91 bp, synthetic construct
  misc_feature 1..91: note = miR30 FDPS sequence #3
  source 1..91: mol_type = other DNA
tgctgttgacagtgagcgactttctcagcctccttctgcgtgaagccacagatggcagaaggaggctgagaaagttgcctactgcctcgga

SEQ ID NO: 8 - DNA, 115 bp, synthetic construct
  misc_feature 1..115: note = miR155 FDPS sequence #1
  source 1..115: mol_type = other DNA
cctggaggcttgctgaaggctgtatgctgactttctcagcctccttctgcttttggccactgactgagcagaagggctgagaaagtcaggacacaaggcctgttactagcactca

SEQ ID NO: 9 - DNA, 114 bp, synthetic construct
  misc_feature 1..114: note = miR21 FDPS sequence #1
  source 1..114: mol_type = other DNA
catctccatggctgtaccaccttgtcgggactttctcagcctccttctgcctgttgaatctcatggcagaaggaggcgagaaagtctgacattttggtatctttcatctgacca

SEQ ID NO: 10 - DNA, 114 bp, synthetic construct
  misc_feature 1..114: note = miR185 FDPS sequence #1
  source 1..114: mol_type = other DNA
gggcctggctcgagcagggggcgagggatactttctcagcctccttctgctggtcccctccccgcagaaggaggctgagaaagtccttccctcccaatgaccgcgtcttcgtcg

SEQ ID NO: 11 - DNA, 228 bp, synthetic construct
  misc_feature 1..228: note = Rous Sarcoma virus (RSV) promoter
  source 1..228: mol_type = other DNA
gtagtcttatgcaatactcttgtagtcttgcaacatggtaacgatgagttagcaacatgccttacaaggagagaaaaagcaccgtgcatgccgattggtggaagtaaggtggtacgatcgtgccttattaggaaggcaacagacgggtctgacatggattggacgaaccactgaattgccgcattgcagagatattgtatttaagtgcctagctcgatacaataaacg

SEQ ID NO: 12 - DNA, 180 bp, synthetic construct
  misc_feature 1..180: note = 5 Long terminal repeat (LTR)
  source 1..180: mol_type = other DNA
ggtctctctggttagaccagatctgagcctgggagctctctggctaactagggaacccactgcttaagcctcaataaagcttgccttgagtgcttcaagtagtgtgtgcccgtctgttgtgtgactctggtaactagagatccctcagacccttttagtcagtgtggaaaatctctagca

SEQ ID NO: 13 - DNA, 41 bp, synthetic construct
  misc_feature 1..41: note = Psi Packaging signal
  source 1..41: mol_type = other DNA
tacgccaaaaattttgactagcggaggctagaaggagagag

SEQ ID NO: 14 - DNA, 233 bp, synthetic construct
  misc_feature 1..233: note = Rev response element (RRE)
  source 1..233: mol_type = other DNA
aggagctttgttccttgggttcttgggagcagcaggaagcactatgggcgcagcctcaatgacgctgacggtacaggccagacaattattgtctggtatagtgcagcagcagaacaatttgctgagggctattgaggcgcaacagcatctgttgcaactcacagtctggggcatcaagcagctccaggcaagaatcctggctgtggaaagatacctaaaggatcaacagctcc

SEQ ID NO: 15 - DNA, 118 bp, synthetic construct
  misc_feature 1..118: note = Central polypurine tract (cPPT)
  source 1..118: mol_type = other DNA
ttttaaaagaaaaggggggattggggggtacagtgcaggggaaagaatagtagacataatagcaacagacatacaaactaaagaattacaaaaacaaattacaaaattcaaaatttta

SEQ ID NO: 16 - DNA, 217 bp, synthetic construct
  misc_feature 1..217: note = Polymerase III shRNA promoters- H1 promoter
  source 1..217: mol_type = other DNA
gaacgctgacgtcatcaacccgctccaaggaatcgcgggcccagtgtcactaggcgggaacacccagcgcgcgtgcgccctggcaggaagatggctgtgagggacaggggagtggcgccctgcaatatttgcatgtcgctatgtgttctgggaaatcaccataaacgtgaaatgtctttggatttgggaatcttataagttctgtatgagaccactt

SEQ ID NO: 17 - DNA, 590 bp, synthetic construct
  misc_feature 1..590: note = Long WPRE sequence
  source 1..590: mol_type = other DNA
aatcaacctctgattacaaaatttgtgaaagattgactggtattcttaactatgttgctccttttacgctatgtggatacgctgctttaatgcctttgtatcatgctattgcttcccgtatggctttcattttctcctccttgtataaatcctggttgctgtctctttatgaggagttgtggcccgttgtcaggcaacgtggcgtggtgtgcactgtgtttgctgacgcaacccccactggttggggcattgccaccacctgtcagctcctttccgggactttcgctttccccctccctattgccacggcggaactcatcgccgcctgccttgcccgctgctggacaggggctcggctgttgggcactgacaattccgtggtgttgtcggggaaatcatcgtcctttccttggctgctcgcctgtgttgccacctggattctgcgcgggacgtccttctgctacgtcccttcggccctcaatccagcggaccttccttcccgcggcctgctgccggctctgcggcctcttccgcgtcttcgccttcgccctcagacgagtcggatctccctttgggccgcctccccgcct

SEQ ID NO: 18 - DNA, 250 bp, synthetic construct
  misc_feature 1..250: note = 3 delta LTR
  source 1..250: mol_type = other DNA
tggaagggctaattcactcccaacgaagataagatctgctttttgcttgtactgggtctctctggttagaccagatctgagcctgggagctctctggctaactagggaacccactgcttaagcctcaataaagcttgccttgagtgcttcaagtagtgtgtgcccgtctgttgtgtgactctggtaactagagatccctcagacccttttagtcagtgtggaaaatctctagcagtagtagttcatgtca

SEQ ID NO: 19 - DNA, 290 bp, synthetic construct
  misc_feature 1..290: note = Helper/Rev- Chicken beta actin (CAG) promoter- Transcription
  source 1..290: mol_type = other DNA
gctattaccatgggtcgaggtgagccccacgttctgcttcactctccccatctcccccccctccccacccccaattttgtatttatttattttttaattattttgtgcagcgatgggggcggggggggggggggcgcgcgccaggcggggcggggcggggcgaggggcggggcggggcgaggcggagaggtgcggcggcagccaatcagagcggcgcgctccgaaagtttccttttatggcgaggcggcggcggcggcggccctataaaaagcgaagcgcgcggcgggcg

SEQ ID NO: 20 - DNA, 1503 bp, synthetic construct
  misc_feature 1..1503: note = Helper/Rev- HIV Gag- Viral capsid
  source 1..1503: mol_type = other DNA
atgggtgcgagagcgtcagtattaagcgggggagaattagatcgatgggaaaaaattcggttaaggccagggggaaagaaaaaatataaattaaaacatatagtatgggcaagcagggagctagaacgattcgcagttaatcctggcctgttagaaacatcagaaggctgtagacaaatactgggacagctacaaccatcccttcagacaggatcagaagaacttagatcattatataatacagtagcaaccctctattgtgtgcatcaaaggatagagataaaagacaccaaggaagctttagacaagatagaggaagagcaaaacaaaagtaagaaaaaagcacagcaagcagcagctgacacaggacacagcaatcaggtcagccaaaattaccctatagtgcagaacatccaggggcaaatggtacatcaggccatatcacctagaactttaaatgcatgggtaaaagtagtagaagagaaggctttcagcccagaagtgatacccatgttttcagcattatcagaaggagccaccccacaagatttaaacaccatgctaaacacagtggggggacatcaagcagccatgcaaatgttaaaagagaccatcaatgaggaagctgcagaatgggatagagtgcatccagtgcatgcagggcctattgcaccaggccagatgagagaaccaaggggaagtgacatagcaggaactactagtacccttcaggaacaaataggatggatgacacataatccacctatcccagtaggagaaatctataaaagatggataatcctgggattaaataaaatagtaagaatgtatagccctaccagcattctggacataagacaaggaccaaaggaaccctttagagactatgtagaccgattctataaaactctaagagccgagcaagcttcacaagaggtaaaaaattggatgacagaaaccttgttggtccaaaatgcgaacccagattgtaagactattttaaaagcattgggaccaggagcgacactagaagaaatgatgacagcatgtcagggagtggggggacccggccataaagcaagagttttggctgaagcaatgagccaagtaacaaatccagctaccataatgatacagaaaggcaattttaggaaccaaagaaagactgttaagtgtttcaattgtggcaaagaagggcacatagccaaaaattgcagggcccctaggaaaaagggctgttggaaatgtggaaaggaaggacaccaaatgaaagattgtactgagagacaggctaattttttagggaagatctggccttcccacaagggaaggccagggaattttcttcagagcagaccagagccaacagccccaccagaagagagcttcaggtttggggaagagacaacaactccctctcagaagcaggagccgatagacaaggaactgtatcctttagcttccctcagatcactctttggcagcgacccctcgtcacaataa

SEQ ID NO: 21 - DNA, 1872 bp, synthetic construct
  misc_feature 1..1872: note = Helper/Rev- HIV Pol- Protease and reverse transcriptase
  source 1..1872: mol_type = other DNA
atgaatttgccaggaagatggaaaccaaaaatgatagggggaattggaggttttatcaaagtaggacagtatgatcagatactcatagaaatctgcggacataaagctataggtacagtattagtaggacctacacctgtcaacataattggaagaaatctgttgactcagattggctgcactttaaattttcccattagtcctattgagactgtaccagtaaaattaaagccaggaatggatggcccaaaagttaaacaatggccattgacagaagaaaaaataaaagcattagtagaaatttgtacagaaatggaaaaggaaggaaaaatttcaaaaattgggcctgaaaatccatacaatactccagtatttgccataaagaaaaaagacagtactaaatggagaaaattagtagatttcagagaacttaataagagaactcaagatttctgggaagttcaattaggaataccacatcctgcagggttaaaacagaaaaaatcagtaacagtactggatgtgggcgatgcatatttttcagttcccttagataaagacttcaggaagtatactgcatttaccatacctagtataaacaatgagacaccagggattagatatcagtacaatgtgcttccacagggatggaaaggatcaccagcaatattccagtgtagcatgacaaaaatcttagagccttttagaaaacaaaatccagacatagtcatctatcaatacatggatgatttgtatgtaggatctgacttagaaatagggcagcatagaacaaaaatagaggaactgagacaacatctgttgaggtggggatttaccacaccagacaaaaaacatcagaaagaacctccattcctttggatgggttatgaactccatcctgataaatggacagtacagcctatagtgctgccagaaaaggacagctggactgtcaatgacatacagaaattagtgggaaaattgaattgggcaagtcagatttatgcagggattaaagtaaggcaattatgtaaacttcttaggggaaccaaagcactaacagaagtagtaccactaacagaagaagcagagctagaactggcagaaaacagggagattctaaaagaaccggtacatggagtgtattatgacccatcaaaagacttaatagcagaaatacagaagcaggggcaaggccaatggacatatcaaatttatcaagagccatttaaaaatctgaaaacaggaaaatatgcaagaatgaagggtgcccacactaatgatgtgaaacaattaacagaggcagtacaaaaaatagccacagaaagcatagtaatatggggaaagactcctaaatttaaattacccatacaaaaggaaacatgggaagcatggtggacagagtattggcaagccacctggattcctgagtgggagtttgtcaatacccctcccttagtgaagttatggtaccagttagagaaagaacccataataggagcagaaactttctatgtagatggggcagccaatagggaaactaaattaggaaaagcaggatatgtaactgacagaggaagacaaaaagttgtccccctaacggacacaacaaatcagaagactgagttacaagcaattcatctagctttgcaggattcgggattagaagtaaacatagtgacagactcacaatatgcattgggaatcattcaagcacaaccagataagagtgaatcagagttagtcagtcaaataatagagcagttaataaaaaaggaaaaagtctacctggcatgggtaccagcacacaaaggaattggaggaaatgaacaagtagatgggttggtcagtgctggaatcaggaaagtacta

SEQ ID NO: 22 - DNA, 867 bp, synthetic construct
  misc_feature 1..867: note = Helper Rev- HIV Integrase- Integration of viral RNA
  source 1..867: mol_type = other DNA
tttttagatggaatagataaggcccaagaagaacatgagaaatatcacagtaattggagagcaatggctagtgattttaacctaccacctgtagtagcaaaagaaatagtagccagctgtgataaatgtcagctaaaaggggaagccatgcatggacaagtagactgtagcccaggaatatggcagctagattgtacacatttagaaggaaaagttatcttggtagcagttcatgtagccagtggatatatagaagcagaagtaattccagcagagacagggcaagaaacagcatacttcctcttaaaattagcaggaagatggccagtaaaaacagtacatacagacaatggcagcaatttcaccagtactacagttaaggccgcctgttggtgggcggggatcaagcaggaatttggcattccctacaatccccaaagtcaaggagtaatagaatctatgaataaagaattaaagaaaattataggacaggtaagagatcaggctgaacatcttaagacagcagtacaaatggcagtattcatccacaattttaaaagaaaaggggggattggggggtacagtgcaggggaaagaatagtagacataatagcaacagacatacaaactaaagaattacaaaaacaaattacaaaaattcaaaattttcgggtttattacagggacagcagagatccagtttggaaaggaccagcaaagctcctctggaaaggtgaaggggcagtagtaatacaagataatagtgacataaaagtagtgccaagaagaaaagcaaagatcatcagggattatggaaaacagatggcaggtgatgattgtgtggcaagtagacaggatgaggattaa

SEQ ID NO: 23 - DNA, 234 bp, synthetic construct
  misc_feature 1..234: note = Helper/Rev- HIV RRE- Binds Rev element
  source 1..234: mol_type = other DNA
aggagctttgttccttgggttcttgggagcagcaggaagcactatgggcgcagcgtcaatgacgctgacggtacaggccagacaattattgtctggtatagtgcagcagcagaacaatttgctgagggctattgaggcgcaacagcatctgttgcaactcacagtctggggcatcaagcagctccaggcaagaatcctggctgtggaaagatacctaaaggatcaacagctcct

SEQ ID NO: 24 - DNA, 351 bp, synthetic construct
  misc_feature 1..351: note = Helper/Rev- HIV Rev- Nuclear export and stabilize viral mRNA
  source 1..351: mol_type = other DNA
atggcaggaagaagcggagacagcgacgaagaactcctcaaggcagtcagactcatcaagtttctctatcaaagcaacccacctcccaatcccgaggggacccgacaggcccgaaggaatagaagaagaaggtggagagagagacagagacagatccattcgattagtgaacggatccttagcacttatctgggacgatctgcggagcctgtgcctcttcagctaccaccgcttgagagacttactcttgattgtaacgaggattgtggaacttctgggacgcagggggtgggaagccctcaaatattggtggaatctcctacaatattggagtcaggagctaaagaatag

SEQ ID NO: 25 - DNA, 577 bp, synthetic construct
  misc_feature 1..577: note = Envelope- CMV promoter- Transcription
  source 1..577: mol_type = other DNA
acattgattattgactagttattaatagtaatcaattacggggtcattagttcatagcccatatatggagttccgcgttacataacttacggtaaatggcccgcctggctgaccgcccaacgacccccgcccattgacgtcaataatgacgtatgttcccatagtaacgccaatagggactttccattgacgtcaatgggtggagtatttacggtaaactgcccacttggcagtacatcaagtgtatcatatgccaagtacgccccctattgacgtcaatgacggtaaatggcccgcctggcattatgcccagtacatgaccttatgggactttcctacttggcagtacatctacgtattagtcatcgctattaccatggtgatgcggttttggcagtacatcaatgggcgtggatagcggtttgactcacggggatttccaagtctccaccccattgacgtcaatgggagtttgttttggcaccaaaatcaacgggactttccaaaatgtcgtaacaactccgccccattgacgcaaatgggcggtaggcgtgtacggtgggaggtctatataagc

SEQ ID NO: 26 - DNA, 1519 bp, synthetic construct
  misc_feature 1..1519: note = Envelope- VSV-G- Glycoprotein envelope-cell entry
  source 1..1519: mol_type = other DNA
atgaagtgccttttgtacttagcctttttattcattggggtgaattgcaagttcaccatagtttttccacacaaccaaaaaggaaactggaaaaatgttccttctaattaccattattgcccgtcaagctcagatttaaattggcataatgacttaataggcacagccttacaagtcaaaatgcccaagagtcacaaggctattcaagcagacggttggatgtgtcatgcttccaaatgggtcactacttgtgatttccgctggtatggaccgaagtatataacacattccatccgatccttcactccatctgtagaacaatgcaaggaaagcattgaacaaacgaaacaaggaacttggctgaatccaggcttccctcctcaaagttgtggatatgcaactgtgacggatgccgaagcagtgattgtccaggtgactcctcaccatgtgctggttgatgaatacacaggagaatgggttgattcacagttcatcaacggaaaatgcagcaattacatatgccccactgtccataactctacaacctggcattctgactataaggtcaaagggctatgtgattctaacctcatttccatggacatcaccttcttctcagaggacggagagctatcatccctgggaaaggagggcacagggttcagaagtaactactttgcttatgaaactggaggcaaggcctgcaaaatgcaatactgcaagcattggggagtcagactcccatcaggtgtctggttcgagatggctgataaggatctctttgctgcagccagattccctgaatgcccagaagggtcaagtatctctgctccatctcagacctcagtggatgtaagtctaattcaggacgttgagaggatcttggattattccctctgccaagaaacctggagcaaaatcagagcgggtcttccaatctctccagtggatctcagctatcttgctcctaaaaacccaggaaccggtcctgctttcaccataatcaatggtaccctaaaatactttgagaccagatacatcagagtcgatattgctgctccaatcctctcaagaatggtcggaatgatcagtggaactaccacagaaagggaactgtgggatgactgggcaccatatgaagacgtggaaattggacccaatggagttctgaggaccagttcaggatataagtttcctttatacatgattggacatggtatgttggactccgatcttcatcttagctcaaaggctcaggtgttcgaacatcctcacattcaagacgctgcttcgcaacttcctgatgatgagagtttattttttggtgatactgggctatccaaaaatccaatcgagcttgtagaaggttggttcagtagttggaaaagctctattgcctcttttttctttatcatagggttaatcattggactattcttggttctccgagttggtatccatctttgcattaaattaaagcacaccaagaaaagacagatttatacagacatagagatga

SEQ ID NO: 27 - DNA, 352 bp, synthetic construct
  misc_feature 1..352: note = Helper/Rev- CMV early (CAG) enhancer- EnhanceTranscription
  source 1..352: mol_type = other DNA
tagttattaatagtaatcaattacggggtcattagttcatagcccatatatggagttccgcgttacataacttacggtaaatggcccgcctggctgaccgcccaacgacccccgcccattgacgtcaataatgacgtatgttcccatagtaacgccaatagggactttccattgacgtcaatgggtggactatttacggtaaactgcccacttggcagtacatcaagtgtatcatatgccaagtacgccccctattgacgtcaatgacggtaaatggcccgcctggcattatgcccagtacatgaccttatgggactttcctacttggcagtacatctacgtattagtcatc

SEQ ID NO: 28 - DNA, 960 bp, synthetic construct
  misc_feature 1..960: note = Helper/Rev- Chicken beta actin intron- Enhance gene expression
  source 1..960: mol_type = other DNA
ggagtcgctgcgttgccttcgccccgtgccccgctccgcgccgcctcgcgccgcccgccccggctctgactgaccgcgttactcccacaggtgagcgggcgggacggcccttctcctccgggctgtaattagcgcttggtttaatgacggctcgtttcttttctgtggctgcgtgaaagccttaaagggctccgggagggccctttgtgcgggggggagcggctcggggggtgcgtgcgtgtgtgtgtgcgtggggagcgccgcgtgcggcccgcgctgcccggcggctgtgagcgctgcgggcgcggcgcggggctttgtgcgctccgcgtgtgcgcgaggggagcgcggccgggggcggtgccccgcggtgcgggggggctgcgaggggaacaaaggctgcgtgcggggtgtgtgcgtgggggggtgagcagggggtgtgggcgcggcggtcgggctgtaacccccccctgcacccccctccccgagttgctgagcacggcccggcttcgggtgcggggctccgtgcggggcgtggcgcggggctcgccgtgccgggcggggggtggcggcaggtgggggtgccgggcggggcggggccgcctcgggccggggagggctcgggggaggggcgcggcggccccggagcgccggcggctgtcgaggcgcggcgagccgcagccattgccttttatggtaatcgtgcgagagggcgcagggacttcctttgtcccaaatctggcggagccgaaatctgggaggcgccgccgcaccccctctagcgggcgcgggcgaagcggtgcggcgccggcaggaaggaaatgggcggggagggccttcgtgcgtcgccgcgccgccgtccccttctccatctccagcctcggggctgccgcagggggacggctgccttcgggggggacggggcagggcggggttcggcttctggcgtgtgaccggcgg

SEQ ID NO: 29 - DNA, 448 bp, synthetic construct
  misc_feature 1..448: note = Helper/Rev- Rabbit beta globin poly A- RNA stability
  source 1..448: mol_type = other DNA
agatctttttccctctgccaaaaattatggggacatcatgaagccccttgagcatctgacttctggctaataaaggaaatttattttcattgcaatagtgtgttggaattttttgtgtctctcactcggaaggacatatgggagggcaaatcatttaaaacatcagaatgagtatttggtttagagtttggcaacatatgccatatgctggctgccatgaacaaaggtggctataaagaggtcatcagtatatgaaacagccccctgctgtccattccttattccatagaaaagccttgacttgaggttagattttttttatattttgttttgtgttatttttttctttaacatccctaaaattttccttacatgttttactagccagatttttcctcctctcctgactactcccagtcatagctgtccctcttctcttatgaagatc

SEQ ID NO: 30 - DNA, 573 bp, synthetic construct
  misc_feature 1..573: note = Envelope- Beta globin intron- Enhance gene expression
  source 1..573: mol_type = other DNA
gtgagtttggggacccttgattgttctttctttttcgctattgtaaaattcatgttatatggagggggcaaagttttcagggtgttgtttagaatgggaagatgtcccttgtatcaccatggaccctcatgataattttgtttctttcactttctactctgttgacaaccattgtctcctcttattttcttttcattttctgtaactttttcgttaaactttagcttgcatttgtaacgaatttttaaattcacttttgtttatttgtcagattgtaagtactttctctaatcacttttttttcaaggcaatcagggtatattatattgtacttcagcacagttttagagaacaattgttataattaaatgataaggtagaatatttctgcatataaattctggctggcgtggaaatattcttattggtagaaacaactacaccctggtcatcatcctgcctttctctttatggttacaatgatatacactgtttgagatgaggataaaatactctgagtccaaaccgggcccctctgctaaccatgttcatgccttcttctctttcctacag

SEQ ID NO: 31 - DNA, 450 bp, synthetic construct
  misc_feature 1..450: note = Envelope- Rabbit beta globin poly A- RNA stability
  source 1..450: mol_type = other DNA
agatctttttccctctgccaaaaattatggggacatcatgaagccccttgagcatctgacttctggctaataaaggaaatttattttcattgcaatagtgtgttggaattttttgtgtctctcactcggaaggacatatgggagggcaaatcatttaaaacatcagaatgagtatttggtttagagtttggcaacatatgcccatatgctggctgccatgaacaaaggttggctataaagaggtcatcagtatatgaaacagccccctgctgtccattccttattccatagaaaagccttgacttgaggttagattttttttatattttgttttgtgttatttttttctttaacatccctaaaattttccttacatgttttactagccagatttttcctcctctcctgactactcccagtcatagctgtccctcttctcttatggagatc

SEQ ID NO: 32 - DNA, 31 bp, synthetic construct
  misc_feature 1..31: note = Primer
  source 1..31: mol_type = other DNA
taagcagaattcatgaatttgccaggaagat

SEQ ID NO: 33 - DNA, 36 bp, synthetic construct
  misc_feature 1..36: note = Primer
  source 1..36: mol_type = other DNA
ccatacaatgaatggacactaggcggccgcacgaat

SEQ ID NO: 34 - DNA, 2745 bp, synthetic construct
  misc_feature 1..2745: note = Gag, Pol, Integrase fragment
  source 1..2745: mol_type = other DNA
gaattcatgaatttgccaggaagatggaaaccaaaaatgatagggggaattggaggttttatcaaagtaagacagtatgatcagatactcatagaaatctgcggacataaagctataggtacagtattagtaggacctacacctgtcaacataattggaagaaatctgttgactcagattggctgcactttaaattttcccattagtcctattgagactgtaccagtaaaattaaagccaggaatggatggcccaaaagttaaacaatggccattgacagaagaaaaaataaaagcattagtagaaatttgtacagaaatggaaaaggaaggaaaaatttcaaaaattgggcctgaaaatccatacaatactccagtatttgccataaagaaaaaagacagtactaaatggagaaaattagtagatttcagagaacttaataagagaactcaagatttctgggaagttcaattaggaataccacatcctgcagggttaaaacagaaaaaatcagtaacagtactggatgtgggcgatgcatatttttcagttcccttagataaagacttcaggaagtatactgcatttaccatacctagtataaacaatgagacaccagggattagatatcagtacaatgtgcttccacagggatggaaaggatcaccagcaatattccagtgtagcatgacaaaaatcttagagccttttagaaaacaaaatccagacatagtcatctatcaatacatggatgatttgtatgtaggatctgacttagaaatagggcagcatagaacaaaaatagaggaactgagacaacatctgttgaggtggggatttaccacaccagacaaaaaacatcagaaagaacctccattcctttggatgggttatgaactccatcctgataaatggacagtacagcctatagtgctgccagaaaaggacagctggactgtcaatgacatacagaaattagtgggaaaattgaattgggcaagtcagatttatgcagggattaaagtaaggcaattatgtaaacttcttaggggaaccaaagcactaacagaagtagtaccactaacagaagaagcagagctagaactggcagaaaacagggagattctaaaagaaccggtacatggagtgtattatgacccatcaaaagacttaatagcagaaatacagaagcaggggcaaggccaatggacatatcaaatttatcaagagccatttaaaaatctgaaaacaggaaagtatgcaagaatgaagggtgcccacactaatgatgtgaaacaattaacagaggcagtacaaaaaatagccacagaaagcatagtaatatggggaaagactcctaaatttaaattacccatacaaaaggaaacatgggaagcatggtggacagagtattggcaagccacctggattcctgagtgggagtttgtcaatacccctcccttagtgaagttatggtaccagttagagaaagaacccataataggagcagaaactttctatgtagatggggcagccaatagggaaactaaattaggaaaagcaggatatgtaactgacagaggaagacaaaaagttgtccccctaacggacacaacaaatcagaagactgagttacaagcaattcatctagctttgcaggattcgggattagaagtaaacatagtgacagactcacaatatgcattgggaatcattcaagcacaaccagataagagtgaatcagagttagtcagtcaaataatagagcagttaataaaaaaggaaaaagtctacctggcatgggtaccagcacacaaaggaattggaggaaatgaacaagtagataaattggtcagtgctggaatcaggaaagtactatttttagatggaatagataaggcccaagaagaacatgagaaatatcacagtaattggagagcaatggctagtgattttaacctaccacctgtagtagcaaaagaaatagtagccagctgtgataaatgtcagctaaaaggggaagccatgcatggacaagtagactgtagcccaggaatatggcagctagattgtacacatttagaaggaaaagttatcttggtagcagttcatgtagccagtggatatatagaagcagaagtaattccagcagagacagggcaagaaacagcatacttcctcttaaaattagcaggaagatggccagtaaaaacagtacatacagacaatggcagcaatttcaccagtactacagttaaggccgcctgttggtgggcggggatcaagcaggaatttggcattccctacaatccccaaagtcaaggagtaatagaatctatgaataaagaattaaagaaaattataggacaggtaagagatcaggctgaacatcttaagacagcagtacaaatggcagtattcatccacaattttaaaagaaaaggggggattggggggtacagtgcaggggaaagaatagtagacataatagcaacagacatacaaactaaagaattacaaaaacaaattacaaaaattcaaaattttcgggtttattacagggacagcagagatccagtttggaaaggaccagcaaagctcctctggaaaggtgaaggggcagtagtaatacaagataatagtgacataaaagtagtgccaagaagaaaagcaaagatcatcagggattatggaaaacagatggcaggtgatgattgtgtggcaagtagacaggatgaggattaa

SEQ ID NO: 35 - DNA, 1586 bp, synthetic construct
  misc_feature 1..1586: note = DNA Fragment containing Rev, RRE and rabbit beta globin poly A
  source 1..1586: mol_type = other DNA
tctagaatggcaggaagaagcggagacagcgacgaagagctcatcagaacagtcagactcatcaagcttctctatcaaagcaacccacctcccaatcccgaggggacccgacaggcccgaaggaatagaagaagaaggtggagagagagacagagacagatccattcgattagtgaacggatccttggcacttatctgggacgatctgcggagcctgtgcctcttcagctaccaccgcttgagagacttactcttgattgtaacgaggattgtggaacttctgggacgcagggggtgggaagccctcaaatattggtggaatctcctacaatattggagtcaggagctaaagaatagaggagctttgttccttgggttcttgggagcagcaggaagcactatgggcgcagcgtcaatgacgctgacggtacaggccagacaattattgtctggtatagtgcagcagcagaacaatttgctgagggctattgaggcgcaacagcatctgttgcaactcacagtctggggcatcaagcagctccaggcaagaatcctggctgtggaaagatacctaaaggatcaacagctcctagatctttttccctctgccaaaaattatggggacatcatgaagccccttgagcatctgacttctggctaataaaggaaatttattttcattgcaatagtgtgttggaattttttgtgtctctcactcggaaggacatatgggagggcaaatcatttaaaacatcagaatgagtatttggtttagagtttggcaacatatgccatatgctggctgccatgaacaaaggtggctataaagaggtcatcagtatatgaaacagccccctgctgtccattccttattccatagaaaagccttgacttgaggttagattttttttatattttgttttgtgttatttttttctttaacatccctaaaattttccttacatgttttactagccagatttttcctcctctcctgactactcccagtcatagctgtccctcttctcttatgaagatccctcgacctgcagcccaagcttggcgtaatcatggtcatagctgtttcctgtgtgaaattgttatccgctcacaattccacacaacatacgagccggaagcataaagtgtaaagcctggggtgcctaatgagtgagctaactcacattaattgcgttgcgctcactgcccgctttccagtcgggaaacctgtcgtgccagcggatccgcatctcaattagtcagcaaccatagtcccgcccctaactccgcccatcccgcccctaactccgcccagttccgcccattctccgccccatggctgactaattttttttatttatgcagaggccgaggccgcctcggcctctgagctattccagaagtagtgaggaggcttttttggaggcctaggcttttgcaaaaagctaacttgtttattgcagcttataatggttacaaataaagcaatagcatcacaaatttcacaaataaagcatttttttcactgcattctagttgtggtttgtccaaactcatcaatgtatcttatcagcggccgccccggg

SEQ ID NO: 36 - DNA, 1614 bp, synthetic construct
  misc_feature 1..1614: note = DNA fragment containing the CAG enhancer/promoter/intron sequence
  source 1..1614: mol_type = other DNA
acgcgttagttattaatagtaatcaattacggggtcattagttcatagcccatatatggagttccgcgttacataacttacggtaaatggcccgcctggctgaccgcccaacgacccccgcccattgacgtcaataatgacgtatgttcccatagtaacgccaatagggactttccattgacgtcaatgggtggactatttacggtaaactgcccacttggcagtacatcaagtgtatcatatgccaagtacgccccctattgacgtcaatgacggtaaatggcccgcctggcattatgcccagtacatgaccttatgggactttcctacttggcagtacatctacgtattagtcatcgctattaccatgggtcgaggtgagccccacgttctgcttcactctccccatctcccccccctccccacccccaattttgtatttatttattttttaattattttgtgcagcgatgggggcggggggggggggggcgcgcgccaggcggggcggggcggggcgaggggcggggcggggcgaggcggagaggtgcggcggcagccaatcagagcggcgcgctccgaaagtttccttttatggcgaggcggcggcggcggcggccctataaaaagcgaagcgcgcggcgggcgggagtcgctgcgttgccttcgccccgtgccccgctccgcgccgcctcgcgccgcccgccccggctctgactgaccgcgttactcccacaggtgagcgggcgggacggcccttctcctccgggctgtaattagcgcttggtttaatgacggctcgtttcttttctgtggctgcgtgaaagccttaaagggctccgggagggccctttgtgcgggggggagcggctcggggggtgcgtgcgtgtgtgtgtgcgtggggagcgccgcgtgcggcccgcgctgcccggcggctgtgagcgctgcgggcgcggcgcggggctttgtgcgctccgcgtgtgcgcgaggggagcgcggccgggggcggtgccccgcggtgcgggggggctgcgaggggaacaaaggctgcgtgcggggtgtgtgcgtgggggggtgagcagggggtgtgggcgcggcggtcgggctgtaacccccccctgcacccccctccccgagttgctgagcacggcccggcttcgggtgcggggctccgtgcggggcgtggcgcggggctcgccgtgccgggcggggggtggcggcaggtgggggtgccgggcggggcggggccgcctcgggccggggagggctcgggggaggggcgcggcggccccggagcgccggcggctgtcgaggcgcggcgagccgcagccattgccttttatggtaatcgtgcgagagggcgcagggacttcctttgtcccaaatctggcggagccgaaatctgggaggcgccgccgcaccccctctagcgggcgcgggcgaagcggtgcggcgccggcaggaaggaaatgggcggggagggccttcgtgcgtcgccgcgccgccgtccccttctccatctccagcctcggggctgccgcagggggacggctgccttcgggggggacggggcagggcggggttcggcttctggcgtgtgaccggcgggaattc

SEQ ID NO: 37 - DNA, 1531 bp, synthetic construct
  misc_feature 1..1531: note = DNA fragment containing VSV-G
  source 1..1531: mol_type = other DNA
gaattcatgaagtgccttttgtacttagcctttttattcattggggtgaattgcaagttcaccatagtttttccacacaaccaaaaaggaaactggaaaaatgttccttctaattaccattattgcccgtcaagctcagatttaaattggcataatgacttaataggcacagccttacaagtcaaaatgcccaagagtcacaaggctattcaagcagacggttggatgtgtcatgcttccaaatgggtcactacttgtgatttccgctggtatggaccgaagtatataacacattccatccgatccttcactccatctgtagaacaatgcaaggaaagcattgaacaaacgaaacaaggaacttggctgaatccaggcttccctcctcaaagttgtggatatgcaactgtgacggatgccgaagcagtgattgtccaggtgactcctcaccatgtgctggttgatgaatacacaggagaatgggttgattcacagttcatcaacggaaaatgcagcaattacatatgccccactgtccataactctacaacctggcattctgactataaggtcaaagggctatgtgattctaacctcatttccatggacatcaccttcttctcagaggacggagagctatcatccctgggaaaggagggcacagggttcagaagtaactactttgcttatgaaactggaggcaaggcctgcaaaatgcaatactgcaagcattggggagtcagactcccatcaggtgtctggttcgagatggctgataaggatctctttgctgcagccagattccctgaatgcccagaagggtcaagtatctctgctccatctcagacctcagtggatgtaagtctaattcaggacgttgagaggatcttggattattccctctgccaagaaacctggagcaaaatcagagcgggtcttccaatctctccagtggatctcagctatcttgctcctaaaaacccaggaaccggtcctgctttcaccataatcaatggtaccctaaaatactttgagaccagatacatcagagtcgatattgctgctccaatcctctcaagaatggtcggaatgatcagtggaactaccacagaaagggaactgtgggatgactgggcaccatatgaagacgtggaaattggacccaatggagttctgaggaccagttcaggatataagtttcctttatacatgattggacatggtatgttggactccgatcttcatcttagctcaaaggctcaggtgttcgaacatcctcacattcaagacgctgcttcgcaacttcctgatgatgagagtttattttttggtgatactgggctatccaaaaatccaatcgagcttgtagaaggttggttcagtagttggaaaagctctattgcctcttttttctttatcatagggttaatcattggactattcttggttctccgagttggtatccatctttgcattaaattaaagcacaccaagaaaagacagatttatacagacatagagatgagaattc

SEQ ID NO: 38 - DNA, 351 bp, synthetic construct; identical to SEQ ID NO: 24
  misc_feature 1..351: note = Rev- RSV promoter- Transcription
  source 1..351: mol_type = other DNA

SEQ ID NO: 39 - DNA, 351 bp, synthetic construct; identical to SEQ ID NO: 24
  misc_feature 1..351: note = Rev- HIV Rev- Nuclear export and stabilize viral mRNA
  source 1..351: mol_type = other DNA

SEQ ID NO: 40 - DNA, 884 bp, synthetic construct
  misc_feature 1..884: note = RSV promoter and HIV Rev
  source 1..884: mol_type = other DNA
caattgcgatgtacgggccagatatacgcgtatctgaggggactagggtgtgtttaggcgaaaagcggggcttcggttgtacgcggttaggagtcccctcaggatatagtagtttcgcttttgcatagggagggggaaatgtagtcttatgcaatacacttgtagtcttgcaacatggtaacgatgagttagcaacatgccttacaaggagagaaaaagcaccgtgcatgccgattggtggaagtaaggtggtacgatcgtgccttattaggaaggcaacagacaggtctgacatggattggacgaaccactgaattccgcattgcagagataattgtatttaagtgcctagctcgatacaataaacgccatttgaccattcaccacattggtgtgcacctccaagctcgagctcgtttagtgaaccgtcagatcgcctggagacgccatccacgctgttttgacctccatagaagacaccgggaccgatccagcctcccctcgaagctagcgattaggcatctcctatggcaggaagaagcggagacagcgacgaagaactcctcaaggcagtcagactcatcaagtttctctatcaaagcaacccacctcccaatcccgaggggacccgacaggcccgaaggaatagaagaagaaggtggagagagagacagagacagatccattcgattagtgaacggatccttagcacttatctgggacgatctgcggagcctgtgcctcttcagctaccaccgcttgagagacttactcttgattgtaacgaggattgtggaacttctgggacgcagggggtgggaagccctcaaatattggtggaatctcctacaatattggagtcaggagctaaagaatagtctaga

SEQ ID NO: 41 - DNA, 1104 bp, synthetic construct
  misc_feature 1..1104: note = Elongation Factor-1 alpha (EF1-alpha) promoter
  source 1..1104: mol_type = other DNA
ccggtgcctagagaaggtggcgcggggtaaactgggaaagtgatgtcgtgtactggctccgcctttttcccgagggtgggggagaaccgtatataagtgcagtagtcgccgtgaacgttctttttcgcaacgggtttgccgccagaacacaggtaagtgccgtgtgtggttcccgcgggcctggcctctttacgggttatggcccttgcgtgccttgaattacttccacgcccctggctgcagtacgtgattcttgatcccgagcttcgggttggaagtgggtgggagagttcgaggccttgcgcttaaggagccccttcgcctcgtgcttgagttgaggcctggcctgggcgctggggccgccgcgtgcgaatctggtggcaccttcgcgcctgtctcgctgctttcgataagtctctagccatttaaaatttttgatgacctgctgcgacgctttttttctggcaagatagtcttgtaaatgcgggccaagatctgcacactggtatttcggtttttggggccgcgggcggcgacggggcccgtgcgtcccagcgcacatgttcggcgaggcggggcctgcgagcgcggccaccgagaatcggacgggggtagtctcaagctggccggcctgctctggtgcctggcctcgcgccgccgtgtatcgccccgccctgggcggcaaggctggcccggtcggcaccagttgcgtgagcggaaagatggccgcttcccggccctgctgcagggagctcaaaatggaggacgcggcgctcgggagagcgggcgggtgagtcacccacacaaaggaaaagggcctttccgtcctcagccgtcgcttcatgtgactccacggagtaccgggcgccgtccaggcacctcgattagttctcgagcttttggagtacgtcgtctttaggttggggggaggggttttatgcgatggagtttccccacactgagtgggtggagactgaagttaggccagcttggcacttgatgtaattctccttggaatttgccctttttgagtttggatcttggttcattctcaagcctcagacagtggttcaaagtttttttcttccatttcaggtgtcgtga

SEQ ID NO: 42 - DNA, 511 bp, synthetic construct
  misc_feature 1..511: note = Promoter- PGK
  source 1..511: mol_type = other DNA
ggggttggggttgcgccttttccaaggcagccctgggtttgcgcagggacgcggctgctctgggcgtggttccgggaaacgcagcggcgccgaccctgggtctcgcacattcttcacgtccgttcgcagcgtcacccggatcttcgccgctacccttgtgggccccccggcgacgcttcctgctccgcccctaagtcgggaaggttccttgcggttcgcggcgtgccggacgtgacaaacggaagccgcacgtctcactagtaccctcgcagacggacagcgccagggagcaatggcagcgcgccgaccgcgatgggctgtggccaatagcggctgctcagcagggcgcgccgagagcagcggccgggaaggggcggtgcgggaggcggggtgtggggcggtagtgtgggccctgttcctgcccgcgcggtgttccgcattctgcaagcctccggagcgcacgtcggcagtcggctccctcgttgaccgaatcaccgacctctctccccag

SEQ ID NO: 43 - DNA, 1162 bp, synthetic construct
  misc_feature 1..1162: note = Promoter- UbC
  source 1..1162: mol_type = other DNA
gcgccgggttttggcgcctcccgcgggcgcccccctcctcacggcgagcgctgccacgtcagacgaagggcgcaggagcgttcctgatccttccgcccggacgctcaggacagcggcccgctgctcataagactcggccttagaaccccagtatcagcagaaggacattttaggacgggacttgggtgactctagggcactggttttctttccagagagcggaacaggcgaggaaaagtagtcccttctcggcgattctgcggagggatctccgtggggcggtgaacgccgatgattatataaggacgcgccgggtgtggcacagctagttccgtcgcagccgggatttgggtcgcggttcttgtttgtggatcgctgtgatcgtcacttggtgagttgcgggctgctgggctggccggggctttcgtggccgccgggccgctcggtgggacggaagcgtgtggagagaccgccaagggctgtagtctgggtccgcgagcaaggttgccctgaactgggggttggggggagcgcacaaaatggcggctgttcccgagtcttgaatggaagacgcttgtaaggcgggctgtgaggtcgttgaaacaaggtggggggcatggtgggcggcaagaacccaaggtcttgaggccttcgctaatgcgggaaagctcttattcgggtgagatgggctggggcaccatctggggaccctgacgtgaagtttgtcactgactggagaactcgggtttgtcgtctggttgcgggggcggcagttatgcggtgccgttgggcagtgcacccgtacctttgggagcgcgcgcctcgtcgtgtcgtgacgtcacccgttctgttggcttataatgcagggtggggccacctgccggtaggtgtgcggtaggcttttctccgtcgcaggacgcagggttcgggcctagggtaggctctcctgaatcgacaggcgccggacctctggtgaggggagggataagtgaggcgtcagtttctttggtcggttttatgtacctatcttcttaagtagctgaagctccggttttgaactatgcgctcggggttggcgagtgtgttttgtgaagttttttaggcaccttttgaaatgtaatcatttgggtcaatatgtaattttcagtgttagactagtaaa

SEQ ID NO: 44 - DNA, 120 bp, synthetic construct
  misc_feature 1..120: note = Poly A- SV40
  source 1..120: mol_type = other DNA
gtttattgcagcttataatggttacaaataaagcaatagcatcacaaatttcacaaataaagcatttttttcactgcattctagttgtggtttgtccaaactcatcaatgtatcttatca

SEQ ID NO: 45 - DNA, 227 bp, synthetic construct
  misc_feature 1..227: note = Poly A- bGH
  source 1..227: mol_type = other DNA
gactgtgccttctagttgccagccatctgttgtttgcccctcccccgtgccttccttgaccctggaaggtgccactcccactgtcctttcctaataaaatgaggaaattgcatcgcattgtctgagtaggtgtcattctattctggggggtggggtggggcaggacagcaagggggaggattgggaagacaatagcaggcatgctggggatgcggtgggctctatgg

SEQ ID NO: 46 - DNA, 1695 bp, synthetic construct
  misc_feature 1..1695: note = Envelope- RD114
  source 1..1695: mol_type = other DNA
atgaaactcccaacaggaatggtcattttatgtagcctaataatagttcgggcagggtttgacgacccccgcaaggctatcgcattagtacaaaaacaacatggtaaaccatgcgaatgcagcggagggcaggtatccgaggccccaccgaactccatccaacaggtaacttgcccaggcaagacggcctacttaatgaccaaccaaaaatggaaatgcagagtcactccaaaaaatctcacccctagcgggggagaactccagaactgcccctgtaacactttccaggactcgatgcacagttcttgttatactgaataccggcaatgcagggcgaataataagacatactacacggccaccttgcttaaaatacggtctgggagcctcaacgaggtacagatattacaaaaccccaatcagctcctacagtccccttgtaggggctctataaatcagcccgtttgctggagtgccacagcccccatccatatctccgatggtggaggacccctcgatactaagagagtgtggacagtccaaaaaaggctagaacaaattcataaggctatgcatcctgaacttcaataccaccccttagccctgcccaaagtcagagatgaccttagccttgatgcacggacttttgatatcctgaataccacttttaggttactccagatgtccaattttagccttgcccaagattgttggctctgtttaaaactaggtacccctacccctcttgcgatacccactccctctttaacctactccctagcagactccctagcgaatgcctcctgtcagattatacctcccctcttggttcaaccgatgcagttctccaactcgtcctgtttatcttcccctttcattaacgatacggaacaaatagacttaggtgcagtcacctttactaactgcacctctgtagccaatgtcagtagtcctttatgtgccctaaacgggtcagtcttcctctgtggaaataacatggcatacacctatttaccccaaaactggacaggactttgcgtccaagcctccctcctccccgacattgacatcatcccgggggatgagccagtccccattcctgccattgatcattatatacatagacctaaacgagctgtacagttcatccctttactagctggactgggaatcaccgcagcattcaccaccggagctacaggcctaggtgtctccgtcacccagtatacaaaattatcccatcagttaatatctgatgtccaagtcttatccggtaccatacaagatttacaagaccaggtagactcgttagctgaagtagttctccaaaataggaggggactggacctactaacggcagaacaaggaggaatttgtttagccttacaagaaaaatgctgtttttatgctaacaagtcaggaattgtgagaaacaaaataagaaccctacaagaagaattacaaaaacgcagggaaagcctggcatccaaccctctctggaccgggctgcagggctttcttccgtacctcctacctctcctgggacccctactcaccctcctactcatactaaccattgggccatgcgttttcaatcgattggtccaatttgttaaagacaggatctcagtggtccaggctctggttttgactcagcaatatcaccagctaaaacccatagagtacgagccatga

SEQ ID NO: 47 - DNA, 2013 bp, synthetic construct
  misc_feature 1..2013: note = Envelope- GALV
  source 1..2013: mol_type = other DNA
atgcttctcacctcaagcccgcaccaccttcggcaccagatgagtcctgggagctggaaaagactgatcatcctcttaagctgcgtattcggagacggcaaaacgagtctgcagaataagaacccccaccagcctgtgaccctcacctggcaggtactgtcccaaactggggacgttgtctgggacaaaaaggcagtccagcccctttggacttggtggccctctcttacacctgatgtatgtgccctggcggccggtcttgagtcctgggatatcccgggatccgatgtatcgtcctctaaaagagttagacctcctgattcagactatactgccgcttataagcaaatcacctggggagccatagggtgcagctaccctcgggctaggaccaggatggcaaattcccccttctacgtgtgtccccgagctggccgaacccattcagaagctaggaggtgtggggggctagaatccctatactgtaaagaatggagttgtgagaccacgggtaccgtttattggcaacccaagtcctcatgggacctcataactgtaaaatgggaccaaaatgtgaaatgggagcaaaaatttcaaaagtgtgaacaaaccggctggtgtaaccccctcaagatagacttcacagaaaaaggaaaactctccagagattggataacggaaaaaacctgggaattaaggttctatgtatatggacacccaggcatacagttgactatccgcttagaggtcactaacatgccggttgtggcagtgggcccagaccctgtccttgcggaacagggacctcctagcaagcccctcactctccctctctccccacggaaagcgccgcccacccctctacccccggcggctagtgagcaaacccctgcggtgcatggagaaactgttaccctaaactctccgcctcccaccagtggcgaccgactctttggccttgtgcagggggccttcctaaccttgaatgctaccaacccaggggccactaagtcttgctggctctgtttgggcatgagccccccttattatgaagggatagcctcttcaggagaggtcgcttatacctccaaccatacccgatgccactggggggcccaaggaaagcttaccctcactgaggtctccggactcgggtcatgcatagggaaggtgcctcttacccatcaacatctttgcaaccagaccttacccatcaattcctctaaaaaccatcagtatctgctcccctcaaaccatagctggtgggcctgcagcactggcctcaccccctgcctctccacctcagtttttaatcagtctaaagacttctgtgtccaggtccagctgatcccccgcatctattaccattctgaagaaaccttgttacaagcctatgacaaatcaccccccaggtttaaaagagagcctgcctcacttaccctagctgtcttcctggggttagggattgcggcaggtataggtactggctcaaccgccctaattaaagggcccatagacctccagcaaggcctaaccagcctccaaatcgccattgacgctgacctccgggcccttcaggactcaatcagcaagctagaggactcactgacttccctatctgaggtagtactccaaaataggagaggccttgacttactattccttaaagaaggaggcctctgcgcggccctaaaagaagagtgctgtttttatgtagaccactcaggtgcagtacgagactccatgaaaaaacttaaagaaagactagataaaagacagttagagcgccagaaaaaccaaaactggtatgaagggtggttcaataactccccttggtttactaccctactatcaaccatcgctgggcccctattgctcctccttttgttactcactcttgggccctgcatcatcaataaattaatccaattcatcaatgataggataagtgcagtcaaaattttagtccttagacagaaatatcagaccctagataacgaggaaaacctttaa

SEQ ID NO: 48 - DNA, 1530 bp, synthetic construct
  misc_feature 1..1530: note = Envelope- FUG
  source 1..1530: mol_type = other DNA
atggttccgcaggttcttttgtttgtactccttctgggtttttcgttgtgtttcgggaagttccccatttacacgataccagacgaacttggtccctggagccctattgacatacaccatctcagctgtccaaataacctggttgtggaggatgaaggatgtaccaacctgtccgagttctcctacatggaactcaaagtgggatacatctcagccatcaaagtgaacgggttcacttgcacaggtgttgtgacagaggcagagacctacaccaactttgttggttatgtcacaaccacattcaagagaaagcatttccgccccaccccagacgcatgtagagccgcgtataactggaagatggccggtgaccccagatatgaagagtccctacacaatccataccccgactaccactggcttcgaactgtaagaaccaccaaagagtccctcattatcatatccccaagtgtgacagatttggacccatatgacaaatcccttcactcaagggtcttccctggcggaaagtgctcaggaataacggtgtcctctacctactgctcaactaaccatgattacaccatttggatgcccgagaatccgagaccaaggacaccttgtgacatttttaccaatagcagagggaagagagcatccaacgggaacaagacttgcggctttgtggatgaaagaggcctgtataagtctctaaaaggagcatgcaggctcaagttatgtggagttcttggacttagacttatggatggaacatgggtcgcgatgcaaacatcagatgagaccaaatggtgccctccagatcagttggtgaatttgcacgactttcgctcagacgagatcgagcatctcgttgtggaggagttagttaagaaaagagaggaatgtctggatgcattagagtccatcatgaccaccaagtcagtaagtttcagacgtctcagtcacctgagaaaacttgtcccagggtttggaaaagcatataccatattcaacaaaaccttgatggaggctgatgctcactacaagtcagtccggacctggaatgagatcatcccctcaaaagggtgtttgaaagttggaggaaggtgccatcctcatgtgaacggggtgtttttcaatggtataatattagggcctgacgaccatgtcctaatcccagagatgcaatcatccctcctccagcaacatatggagttgttggaatcttcagttatccccctgatgcaccccctggcagacccttctacagttttcaaagaaggtgatgaggctgaggattttgttgaagttcacctccccgatgtgtacaaacagatctcaggggttgacctgggtctcccgaactggggaaagtatgtattgatgactgcaggggccatgattggcctggtgttgatattttccctaatgacatggtgcagagttggtatccatctttgcattaaattaaagcacaccaagaaaagacagatttatacagacatagagatgaaccgacttggaaagtaa

SEQ ID NO: 49 - DNA, 1497 bp, synthetic construct
  misc_feature 1..1497: note = Envelope- LCMV
  source 1..1497: mol_type = other DNA
atgggtcagattgtgacaatgtttgaggctctgcctcacatcatcgatgaggtgatcaacattgtcattattgtgcttatcgtgatcacgggtatcaaggctgtctacaattttgccacctgtgggatattcgcattgatcagtttcctacttctggctggcaggtcctgtggcatgtacggtcttaagggacccgacatttacaaaggagtttaccaatttaagtcagtggagtttgatatgtcacatctgaacctgaccatgcccaacgcatgttcagccaacaactcccaccattacatcagtatggggacttctggactagaattgaccttcaccaatgattccatcatcagtcacaacttttgcaatctgacctctgccttcaacaaaaagacctttgaccacacactcatgagtatagtttcgagcctacacctcagtatcagagggaactccaactataaggcagtatcctgcgacttcaacaatggcataaccatccaatacaacttgacattctcagatcgacaaagtgctcagagccagtgtagaaccttcagaggtagagtcctagatatgtttagaactgccttcggggggaaatacatgaggagtggctggggctggacaggctcagatggcaagaccacctggtgtagccagacgagttaccaatacctgattatacaaaatagaacctgggaaaaccactgcacatatgcaggtccttttgggatgtccaggattctcctttcccaagagaagactaagttcttcactaggagactagcgggcacattcacctggactttgtcagactcttcaggggtggagaatccaggtggttattgcctgaccaaatggatgattcttgctgcagagcttaagtgtttcgggaacacagcagttgcgaaatgcaatgtaaatcatgatgccgaattctgtgacatgctgcgactaattgactacaacaaggctgctttgagtaagttcaaagaggacgtagaatctgccttgcacttattcaaaacaacagtgaattctttgatttcagatcaactactgatgaggaaccacttgagagatctgatgggggtgccatattgcaattactcaaagttttggtacctagaacatgcaaagaccggcgaaactagtgtccccaagtgctggcttgtcaccaatggttcttacttaaatgagacccacttcagtgatcaaatcgaacaggaagccgataacatgattacagagatgttgaggaaggattacataaagaggcaggggagtacccccctagcattgatggaccttctgatgttttccacatctgcatatctagtcagcatcttcctgcaccttgtcaaaataccaacacacaggcacataaaaggtggctcatgtccaaagccacaccgattaaccaacaaaggaatttgtagttgtggtgcatttaaggtgcctggtgtaaaaaccgtctggaaaagacgctga

SEQ ID NO: 50 - DNA, 1692 bp, synthetic construct
  misc_feature 1..1692: note = Envelope- FPV
  source 1..1692: mol_type = other DNA
atgaacactcaaatcctggttttcgcccttgtggcagtcatccccacaaatgcagacaaaatttgtcttggacatcatgctgtatcaaatggcaccaaagtaaacacactcactgagagaggagtagaagttgtcaatgcaacggaaacagtggagcggacaaacatccccaaaatttgctcaaaagggaaaagaaccactgatcttggccaatgcggactgttagggaccattaccggaccacctcaatgcgaccaatttctagaattttcagctgatctaataatcgagagacgagaaggaaatgatgtttgttacccggggaagtttgttaatgaagaggcattgcgacaaatcctcagaggatcaggtgggattgacaaagaaacaatgggattcacatatagtggaataaggaccaacggaacaactagtgcatgtagaagatcagggtcttcattctatgcagaaatggagtggctcctgtcaaatacagacaatgctgctttcccacaaatgacaaaatcatacaaaaacacaaggagagaatcagctctgatagtctggggaatccaccattcaggatcaaccaccgaacagaccaaactatatgggagtggaaataaactgataacagtcgggagttccaaatatcatcaatcttttgtgccgagtccaggaacacgaccgcagataaatggccagtccggacggattgattttcattggttgatcttggatcccaatgatacagttacttttagtttcaatggggctttcatagctccaaatcgtgccagcttcttgaggggaaagtccatggggatccagagcgatgtgcaggttgatgccaattgcgaaggggaatgctaccacagtggagggactataacaagcagattgccttttcaaaacatcaatagcagagcagttggcaaatgcccaagatatgtaaaacaggaaagtttattattggcaactgggatgaagaacgttcccgaaccttccaaaaaaaggaaaaaaagaggcctgtttggcgctatagcagggtttattgaaaatggttgggaaggtctggtcgacgggtggtacggtttcaggcatcagaatgcacaaggagaaggaactgcagcagactacaaaagcacccaatcggcaattgatcagataaccggaaagttaaatagactcattgagaaaaccaaccagcaatttgagctaatagataatgaattcactgaggtggaaaagcagattggcaatttaattaactggaccaaagactccatcacagaagtatggtcttacaatgctgaacttcttgtggcaatggaaaaccagcacactattgatttggctgattcagagatgaacaagctgtatgagcgagtgaggaaacaattaagggaaaatgctgaagaggatggcactggttgctttgaaatttttcataaatgtgacgatgattgtatggctagtataaggaacaatacttatgatcacagcaaatacagagaagaagcgatgcaaaatagaatacaaattgacccagtcaaattgagtagtggctacaaagatgtgatactttggtttagcttcggggcatcatgctttttgcttcttgccattgcaatgggccttgttttcatatgtgtgaagaacggaaacatgcggtgcactatttgtatataa

SEQ ID NO: 51 - DNA, 1266 bp, synthetic construct
  misc_feature 1..1266: note = Envelope- RRV
  source 1..1266: mol_type = other DNA
agtgtaacagagcactttaatgtgtataaggctactagaccatacctagcacattgcgccgattgcggggacgggtacttctgctatagcccagttgctatcgaggagatccgagatgaggcgtctgatggcatgcttaagatccaagtctccgcccaaataggtctggacaaggcaggcacccacgcccacacgaagctccgatatatggctggtcatgatgttcaggaatctaagagagattccttgagggtgtacacgtccgcagcgtgctccatacatgggacgatgggacacttcatcgtcgcacactgtccaccaggcgactacctcaaggtttcgttcgaggacgcagattcgcacgtgaaggcatgtaaggtccaatacaagcacaatccattgccggtgggtagagagaagttcgtggttagaccacactttggcgtagagctgccatgcacctcataccagctgacaacggctcccaccgacgaggagattgacatgcatacaccgccagatataccggatcgcaccctgctatcacagacggcgggcaacgtcaaaataacagcaggcggcaggactatcaggtacaactgtacctgcggccgtgacaacgtaggcactaccagtactgacaagaccatcaacacatgcaagattgaccaatgccatgctgccgtcaccagccatgacaaatggcaatttacctctccatttgttcccagggctgatcagacagctaggaaaggcaaggtacacgttccgttccctctgactaacgtcacctgccgagtgccgttggctcgagcgccggatgccacctatggtaagaaggaggtgaccctgagattacacccagatcatccgacgctcttctcctataggagtttaggagccgaaccgcacccgtacgaggaatgggttgacaagttctctgagcgcatcatcccagtgacggaagaagggattgagtaccagtggggcaacaacccgccggtctgcctgtgggcgcaactgacgaccgagggcaaaccccatggctggccacatgaaatcattcagtactattatggactataccccgccgccactattgccgcagtatccggggcgagtctgatggccctcctaactctggcggccacatgctgcatgctggccaccgcgaggagaaagtgcctaacaccgtacgccctgacgccaggagcggtggtaccgttgacactggggctgctttgctgcgcaccgagggcgaatgca

SEQ ID NO: 52 - DNA, 1266 bp, synthetic construct; identical to SEQ ID NO: 51
  misc_feature 1..1266: note = Envelope- MLV 10A1
  source 1..1266: mol_type = other DNA

SEQ ID NO: 53 - DNA, 2030 bp, synthetic construct
  misc_feature 1..2030: note = Envelope- Ebola
  source 1..2030: mol_type = other DNA
atgggtgttacaggaatattgcagttacctcgtgatcgattcaagaggacatcattctttctttgggtaattatccttttccaaagaacattttccatcccacttggagtcatccacaatagcacattacaggttagtgatgtcgacaaactggtttgccgtgacaaactgtcatccacaaatcaattgagatcagttggactgaatctcgaagggaatggagtggcaactgacgtgccatctgcaactaaaagatggggcttcaggtccggtgtcccaccaaaggtggtcaattatgaagctggtgaatgggctgaaaactgctacaatcttgaaatcaaaaaacctgacgggagtgagtgtctaccagcagcgccagacgggattcggggcttcccccggtgccggtatgtgcacaaagtatcaggaacgggaccgtgtgccggagactttgccttccacaaagagggtgctttcttcctgtatgaccgacttgcttccacagttatctaccgaggaacgactttcgctgaaggtgtcgttgcatttctgatactgccccaagctaagaaggacttcttcagctcacaccccttgagagagccggtcaatgcaacggaggacccgtctagtggctactattctaccacaattagatatcaagctaccggttttggaaccaatgagacagagtatttgttcgaggttgacaatttgacctacgtccaacttgaatcaagattcacaccacagtttctgctccagctgaatgagacaatatatacaagtgggaaaaggagcaataccacgggaaaactaatttggaaggtcaaccccgaaattgatacaacaatcggggagtgggccttctgggaaactaaaaaaacctcactagaaaaattcgcagtgaagagttgtctttcacagctgtatcaaacagagccaaaaacatcagtggtcagagtccggcgcgaacttcttccgacccagggaccaacacaacaactgaagaccacaaaatcatggcttcagaaaattcctctgcaatggttcaagtgcacagtcaaggaagggaagctgcagtgtcgcatctgacaacccttgccacaatctccacgagtcctcaaccccccacaaccaaaccaggtccggacaacagcacccacaatacacccgtgtataaacttgacatctctgaggcaactcaagttgaacaacatcaccgcagaacagacaacgacagcacagcctccgacactccccccgccacgaccgcagccggacccctaaaagcagagaacaccaacacgagcaagggtaccgacctcctggaccccgccaccacaacaagtccccaaaaccacagcgagaccgctggcaacaacaacactcatcaccaagataccggagaagagagtgccagcagcgggaagctaggcttaattaccaatactattgctggagtcgcaggactgatcacaggcgggaggagagctcgaagagaagcaattgtcaatgctcaacccaaatgcaaccctaatttacattactggactactcaggatgaaggtgctgcaatcggactggcctggataccatatttcgggccagcagccgagggaatttacatagaggggctgatgcacaatcaagatggtttaatctgtgggttgagacagctggccaacgagacgactcaagctcttcaactgttcctgagagccacaaccgagctacgcaccttttcaatcctcaaccgtaaggcaattgatttcttgctgcagcgatggggcggcacatgccacattttgggaccggactgctgtatcgaaccacatgattggaccaagaacataacagacaaaattgatcagattattcatgattttgttgataaaacccttccggaccagggggacaatgacaattggtggacaggatggagacaatggataccggcaggtattggagttacaggcgttataattgcagttatcgctttattctgtatatgcaaatttgtcttttag

SEQ ID NO: 54 - DNA, 237 bp, synthetic construct
  misc_feature 1..237: note = Polymerase III shRNA promoters- U6 promoter
  source 1..237: mol_type = other DNA
tttcccatgattccttcatatttgcatatacgatacaaggctgttagagagataattggaattaatttgactgtaaacacaaagatattagtacaaaatacgtgacgtagaaagtaataatttcttgggtagtttgcagttttaaaattatgttttaaaatggactatcatatgcttaccgtaacttgaaagtatttcgatttcttggctttatatatcttgtggaaaggacgaaac

SEQ ID NO: 55 - DNA, 243 bp, synthetic construct
  misc_feature 1..243: note = Polymerase III shRNA promoters- 7SK promoter
  source 1..243: mol_type = other DNA
ctgcagtatttagcatgccccacccatctgcaaggcattctggatagtgtcaaaacagccggaaatcaagtccgtttatctcaaactttagcattttgggaataaatgatatttgctatgctggttaaattagattttagttaaatttcctgctgaagctctagtacgataagcaacttgacctaagtgtaaagttgagatttccttcaggtttatatagcttgtgcgccgcctggctacctc

SEQ ID NO: 56 - DNA, 21 bp, synthetic construct
  misc_feature 1..21: note = FDPS target sequence #1
  source 1..21: mol_type = other DNA
gtcctggagtacaatgccatt

SEQ ID NO: 57 - DNA, 21 bp, synthetic construct
  misc_feature 1..21: note = FDPS target sequence #2
  source 1..21: mol_type = other DNA
gcaggatttcgttcagcactt

SEQ ID NO: 58 - DNA, 21 bp, synthetic construct
  misc_feature 1..21: note = FDPS target sequence #3
  source 1..21: mol_type = other DNA
gccatgtacatggcaggaatt

SEQ ID NO: 59 - DNA, 21 bp, synthetic construct
  misc_feature 1..21: note = FDPS target sequence #4
  source 1..21: mol_type = other DNA
gcagaaggaggctgagaaagt

SEQ ID NO: 60 - DNA, 49 bp, synthetic construct
  misc_feature 1..49: note = Non-targeting sequence
  source 1..49: mol_type = other DNA
gccgctttgtaggatagagctcgagctctatcctacaaagcggcttttt

SEQ ID NO: 61 - DNA, 20 bp, synthetic construct
  misc_feature 1..20: note = Forward primer
  source 1..20: mol_type = other DNA
aggaattgatggcgagaagg

SEQ ID NO: 62 - DNA, 22 bp, synthetic construct
  misc_feature 1..22: note = Reverse primer
  source 1..22: mol_type = other DNA
cccaaagaggtcaaggtaatca

SEQ ID NO: 63 - DNA, 18 bp, synthetic construct
  misc_feature 1..18: note = Forward primer
  source 1..18: mol_type = other DNA
agcgcggctacagcttca

SEQ ID NO: 64 - DNA, 20 bp, synthetic construct
  misc_feature 1..20: note = Reverse primer
  source 1..20: mol_type = other DNA
ggcgacgtagcacagcttct

SEQ ID NO: 65 - DNA, 130 bp, synthetic construct
  misc_feature 1..130: note = Left Inverted Terminal Repeat (Left ITR)
  source 1..130: mol_type = other DNA
cctgcaggcagctgcgcgctcgctcgctcactgaggccgcccgggcgtcgggcgacctttggtcgcccggcctcagtgagcgagcgagcgcgcagagagggagtggccaactccatcactaggggttcct

SEQ ID NO: 66 - DNA, 151 bp, synthetic construct
  misc_feature 1..151: note = Right Inverted Terminal Repeat (Right ITR)
  source 1..151: mol_type = other DNA
gagcggccgcaggaacccctagtgatggagttggccactccctctctgcgcgctcgctcgctcactgaggccgggcgaccaaaggtcgcccgacgcccgggctttgcccgggcggcctcagtgagcgagcgagcgcgcagctgcctgcagg

SEQ ID NO: 67 - DNA, 1227 bp, synthetic construct
  misc_feature 1..1227: note = Helper plasmid without REV
  source 1..1227: mol_type = other DNA
tctagaaggagctttgttccttgggttcttgggagcagcaggaagcactatgggcgcagcgtcaatgacgctgacggtacaggccagacaattattgtctggtatagtgcagcagcagaacaatttgctgagggctattgaggcgcaacagcatctgttgcaactcacagtctggggcatcaagcagctccaggcaagaatcctggctgtggaaagatacctaaaggatcaacagctcctagatctttttccctctgccaaaaattatggggacatcatgaagccccttgagcatctgacttctggctaataaaggaaatttattttcattgcaatagtgtgttggaattttttgtgtctctcactcggaaggacatatgggagggcaaatcatttaaaacatcagaatgagtatttggtttagagtttggcaacatatgccatatgctggctgccatgaacaaaggtggctataaagaggtcatcagtatatgaaacagccccctgctgtccattccttattccatagaaaagccttgacttgaggttagattttttttatattttgttttgtgttatttttttctttaacatccctaaaattttccttacatgttttactagccagatttttcctcctctcctgactactcccagtcatagctgtccctcttctcttatgaagatccctcgacctgcagcccaagcttggcgtaatcatggtcatagctgtttcctgtgtgaaattgttatccgctcacaattccacacaacatacgagccggaagcataaagtgtaaagcctggggtgcctaatgagtgagctaactcacattaattgcgttgcgctcactgcccgctttccagtcgggaaacctgtcgtgccagcggatccgcatctcaattagtcagcaaccatagtcccgcccctaactccgcccatcccgcccctaactccgcccagttccgcccattctccgccccatggctgactaattttttttatttatgcagaggccgaggccgcctcggcctctgagctattccagaagtagtgaggaggcttttttggaggcctaggcttttgcaaaaagctaacttgtttattgcagcttataatggttacaaataaagcaatagcatcacaaatttcacaaataaagcatttttttcactgcattctagttgtggtttgtccaaactcatcaatgtatcttatcacccggg